European Patent Application EP 4 245 842 A1, published September 20, 2023. Title: Composition for controlling plant disease comprising culture solution of Streptomyces sp. Strain or extract thereof, and controlling method for plant disease. Applicant: INDUSTRY FOUNDATION OF CHONNAM NATIONAL UNIVERSITY. The sequence listing filed with the application follows.

SEQUENCE LISTING (3 sequences)

SEQ ID NO: 1 - DNA, 18 bp, Artificial Sequence
  JCK-6141 16S rRNA 9F forward primer
gagtttgatcctggctca

SEQ ID NO: 2 - DNA, 21 bp, Artificial Sequence
  JCK-6141 16S rRNA 1512R reverse primer
acggctaccttgttacgactt

SEQ ID NO: 3 - DNA, 1338 bp, Streptomyces sp.
ggattagtggcgaacgggtgagtaacacgtgggcaatctgcccttcactctgggacaagccctggaaacggggtctaataccggatatgagcctgggaggcatctcccgggttgtaaagctccggcggtgaaggatgagcccgcggcctatcagcttgttggtgaggtaatggctcaccaaggcgacgacgggtagccggcctgagagggcgaccggccacactgggactgagacacggcccagactcctacgggaggcagcagtggggaatattgcacaatgggcgaaagcctgatgcagcgacgccgcgtgagggatgacggccttcgggttgtaaacctctttcagcagggaagaagcgaaagtgacggtacctgcagaagaagcgccggctaactacgtgccagcagccgcggtaatacgtagggcgcaagcgttgtccggaattattgggcgtaaagagctcgtaggcggcttgtcacgtcgattgtgaaagcccgaggcttaacctcgggtctgcagtcgatacgggctagctagagtgtggtaggggagatcggaattcctggtgtagcggtgaaatgcgcagatatcaggaggaacaccggtggcgaaggcggatctctgggccattactgacgctgaggagcgaaagcgtggggagcgaacaggattagataccctggtagtccacgccgtaaacggtgggaactaggtgttggcgacattccacgtcgtcggtgccgcagctaacgcattaagttccccgcctggggagtacggccgcaaggctaaaactcaaaggaattgacgggggcccgcacaagcggcggagcatgtggcttaattcgacgcaacgcgaagaaccttaccaaggcttgacatacaccggaaagcattagagatagtgccccccttgtggtcggtgtacaggtggtgcatggctgtcgtcagctcgtgtcgtgagatgttgggttaagtcccgcaacgagcgcaacccttgttctgtgttgccagcatgcccttcggggtgatggggactcacaggagaccgccggggtcaactcggaggaaggtggggacgacgtcaagtcatcatgccccttatgtcttgggctgcacacgtgctacaatggccggtacaatgagctgcgataccgtgaggtggagcgaatctcaaaaagccggtctcagttcggattggggtctgcaactcgaccccatgaagtcggagtcgctagtaatcgcagatcagcattgctgcggtgaatacgttcccgggccttgtacacaccgcccgtcacgtcacgaaagtcggtaacacccgaagccggtgg